European Patent Application EP 4 692 352 A1, published February 11, 2026. Title: Method for producing fish, fish and method for producing fish gametes. Applicant: Tokyo University of Marine Science and Technology. The sequence listing filed with the application follows.

SEQUENCE LISTING (26 sequences)

SEQ ID NO: 1 - DNA, 411 bp, Oncorhynchus mykiss
  source 1..411: mol_type = other DNA
atgtactgcacccacttaaagatgctgcagctggtcgtcatggcaacgctgtgggtgacaccagtgagggcggggacagactgcaggtatggctgccgactaaacaacatgaccatcaccgtggagagagaggactgtcacggaagcatcaccgtcaccacctgcgccggcctgtgcgaaacaacggacctgaactatcagagcacatggctgccgcgctcccagggggtgtgtaacttcaaggagtggtcctacgagaaggtctacctggaaggctgtccatccggggtcaaccccctcttcatacccgttgccaagagctgcgattgcatcaaatgcaagacggacaacaccgactgtgatcgcataagcatggcaacacccagctgcatagtaaacccactagaaatg

SEQ ID NO: 2 - DNA, 279 bp, Oncorhynchus mykiss
  source 1..279: mol_type = other DNA
tatccaaacagtgacaagacaaacatgggctgtgaggaatgcacactgaagccgaacacaatcttccccaacatcatgcagtgtacaggctgttgcttctccagagcttatccaaccccactacggtccaagcaaaccatgctggttcccaagaacatcacctctgaagccacatgctgcgttgcaaaagaaggggaaagggtcaccaccaaggatggcttcccggtgacgaaccacacagagtgtcactgcagcacctgctattaccataaatcataa

SEQ ID NO: 3 - DNA, 123 bp, Oncorhynchus mykiss
  source 1..123: mol_type = other DNA
tcctcttcctctaaggatccacatcaccatcaccatcacccatcccaacctctcacatccacatccaccccaactcctggggccagcagacgttcctctcatcccctcccaataaagacttct

SEQ ID NO: 4 - DNA, 35 bp, synthetic construct
  source 1..35: mol_type = other DNA
gtaccgggccccccctcgagcgcaaccaagggcta

SEQ ID NO: 5 - DNA, 35 bp, synthetic construct
  source 1..35: mol_type = other DNA
cccccgggctgcaggaattctcccttagacatgtt

SEQ ID NO: 6 - DNA, 38 bp, synthetic construct
  source 1..38: mol_type = other DNA
ggtaccgggccccccctcgagatgttaggtcttcatgt

SEQ ID NO: 7 - DNA, 35 bp, synthetic construct
  source 1..35: mol_type = other DNA
ggtaccgggccccccctcgagaagcttgtttatta

SEQ ID NO: 8 - DNA, 26 bp, synthetic construct
  source 1..26: mol_type = other DNA
acattccattgtttctgcaactacct

SEQ ID NO: 9 - DNA, 39 bp, synthetic construct
  source 1..39: mol_type = other DNA
tcccccgggctgcaggaattcaagcttgtttattaaact

SEQ ID NO: 10 - DNA, 49 bp, synthetic construct
  source 1..49: mol_type = other DNA
ggtaccgggccccccctcgagcgcaaccaagggctagcaatgtcagtaa

SEQ ID NO: 11 - DNA, 35 bp, synthetic construct
  source 1..35: mol_type = other DNA
cctacatgaagacctaacattcccttagacatgtt

SEQ ID NO: 12 - DNA, 25 bp, synthetic construct
  source 1..25: mol_type = other DNA
atgttaggtcttcatgtaggcacct

SEQ ID NO: 13 - DNA, 111 bp, synthetic construct
  source 1..111: mol_type = other DNA
tcctcttcctctaaggatccacatcaccatcaccatcacccatcccaacctctcacatccacatccaccccaactcctggggccagcagacgttcctctcatcccctccca

SEQ ID NO: 14 - DNA, 25 bp, synthetic construct
  source 1..25: mol_type = other DNA
tcccttagacatgttacctggacaa

SEQ ID NO: 15 - DNA, 35 bp, synthetic construct
  source 1..35: mol_type = other DNA
caggtaacatgtctaagggaatgtactgcacccac

SEQ ID NO: 16 - DNA, 35 bp, synthetic construct
  source 1..35: mol_type = other DNA
ggatccttagaggaagaggacatttctagtgggtt

SEQ ID NO: 17 - DNA, 22 bp, synthetic construct
  source 1..22: mol_type = other DNA
tcaaccccctcttcatacccgt

SEQ ID NO: 18 - DNA, 20 bp, synthetic construct
  source 1..20: mol_type = other DNA
accctttccccttcttttgc

SEQ ID NO: 19 - protein, 137 aa, Oncorhynchus mykiss
MYCTHLKMLQLVVMATLWVTPVRAGTDCRYGCRLNNMTITVEREDCHGSITVTTCAGLCETTDLNYQSTWLPRSQGVCNFKEWSYEKVYLEGCPSGVNPLFIPVAKSCDCIKCKTDNTDCDRISMATPSCIVNPLEM

SEQ ID NO: 20 - protein, 92 aa, Oncorhynchus mykiss
YPNSDKTNMGCEECTLKPNTIFPNIMQCTGCCFSRAYPTPLRSKQTMLVPKNITSEATCCVAKEGERVTTKDGFPVTNHTECHCSTCYYHKS

SEQ ID NO: 21 - DNA, 2836 bp, Oncorhynchus mykiss
  source 1..2836: mol_type = genomic DNA
cgcaaccaagggctagcaatgtcagtaaagctagtcacctggaccacgagttgccgaagctcgttcagtgtttcagagttaaaaaatgtgttttaaataatttaagaactgcaaatgcaatgctcacttataatttaataattacaattttgcttcctatggcgggcaagggaggtctggttgtcggccatgctggaaatgtgatctcgcgttattgtgccattgtcaatacagtacatctacaccacgatatgaaacgttgatttgaaccttctgactcacttgtgaatcagacgggccccatggtctgatttaaatcgcatgatatctgatgatagttgtcgaatatatcgactgattgcattacctcatccccatactgtatttatttatttatcttgctcctttgcacctcagtatctctacttgcacattcatcttctgcacatctaacattccagtgtttaattgctatattgtaattacttcgccaccatggcctatttattgccttaacgctcttatcttacctcatttgcactcactgcattctttttctactgtattattgactgtatgttttgtttattccatgtgtaactctgtgttgttgtaaatgtcgaactgctatgatttatcttggccaggtcgcagttgcaaatgagaacttgttctcaactaacctacctggttaaataaaggttaaataaaggttaaataaaaaataaataaataaaaagtgtatccggtgcgaacgcaacccgacgtcttcatgggaagtgggagggagcaacagcctgtgtttttattggtattttggaatgtcaagttgaatcctgagctatgattggttgccttgccgtttatatagtaatggtagacttatccttccttctttctctcacaacacacaaggcgaagaaagggaggcttcgccattgttcaactccgatcaacatcagcatcaccttcggtcaaataatttattcggtaagtaagaactagtttaatttaatagtaatgtaataatgaaagcgtttttttttagttcaccgtaatttattttgctgaccacaagccggtacattttatatccggaagacaaggctggctaacgtaaattaactacttggccttgtagttttaactaatatcacctagtcgacaaattaaaccttgtaaaacttacctaactgatctagctttaactcggaattactgcaatatatttacatgttctatcctatttgatatcatttaactgttaacgttgggcaactagttcgcttttagttggcctttgcttgctaactaatcggtcaacctttaatgtcgtggttaatatcacagctaataattatttgattgacattcgatcgacagtttcaaacagtttttgtcactgcgctaggtaacaacggttgtatgcggtataccaggatatggcgcgcgaccaccctcgtggtcggcctagttctagaacgttctagagactctgcaccccgcgtgatgtgacgcacaaaaggacgtccgttgttctttctgaagtgtaataccggtacataccggtatctgttgctgaagttggtgtcgacgtgagcaccgtatcttgaattaaaccgttttattggttagtcgatactttagttttgctgaccttattctcataggctgttcgggggacaaatatttaactttggttgtgttatatcttatgatctctttatagcgatcactattttgagcgaaggacttaaaataagggaagtttattgtttttctagtcaatggtatcaaatcaattgaattaactttttgggcgacctgacggtaattcgcatgcgagttatagagctctcattgaaagtcttaaaagcggtaggtctgatataggtgcgccatttctatgtttccgggtcacaagcttctttctgcttctactttctattttctgaaagtattttcggctttggaaaataatttagtagtttcgatggtgcgaccggtctaccctatagctgttgcataaactgtatttgggaaaatatcagttttggcaaccaggaaatggctgcggtttatgcttagtggctttaaatttaacttgatagtatttcaaaccactaattgactgactttggttcaattatttgaggaatattttcccctgtgagctcagtgcgctcgctgccgtttcttgggtgaaatcagatccagcctgaactgtgccatgtagtgggtagtttgtaacttccaactggccaatttcctacacatttgagaacatgtggtaattaactacaatgactaattggttatctacatttatccctgcccctgaggcaaatggcactatggagtgcctgaggtggcaaaatgtaaatctggaactatccctgacaaccaatgtcaatgtagctacagggttcaacttcgtagaatgatttcatgtctcggaacaatgacaggagtggaggtgttttgctttttcggtgaagatgtcaaatgaccatcaaacaaaatcaggactctaccatactacttgacaatacaatgtcgcatcaatcttactcggttaggttgaagaataccattgtgaatgtgaacacgaatttagcagttttcaaagacctgtcccacattggaaaattcctaggatggtacttgagtctacaatgtgcagttgggcctagaggggtaactaatgtttacaaatgaccaatgtattttgatgaccacattggcttctagctgatatttttactgcgtttgttgtattcttgcatagtgtccatttgttacctaacaccatgctgttcttcattgtccaggtaac

SEQ ID NO: 22 - DNA, 12 bp, Oncorhynchus mykiss
  source 1..12: mol_type = genomic DNA
atgtctaaggga

SEQ ID NO: 23 - DNA, 660 bp, Oncorhynchus mykiss
  source 1..660: mol_type = genomic DNA
acattccattgtttctgcaactacctccccctaacaagcaaagtttgaaatgtgttctaccctcttgtgtctgagtctcgtgacttgtcaaggagtgaaatttgaataaaggttgggggatcacatatttttcaactttgtttgctacgcaacagggaacagtaattttctgttagcacaactaagctgtcaaatttcacatgtgtattttctcagttgtcatctgcctttgtcacaatgcctttaggacaaaataaaatatacggtgaccttccacctttacttctaaatgtttgggtcctttacactactttggaaaagggaagatgttaggaagggccatattttggtcaatattgtcatgacaaagttcaatattgcttgtagcttcccacaaacttccagctgctagaccagtgtaaagatgtcttgaggtcctgcgtccattcatacctgaccctttttttttgaatgtggtagtgcttcatatctataccattggaaaaacataaattgctttaagtgactaccgagtcattttggtacatttcctcgtgtgcctaaccaaagcaaaaaaggccctggcctatggaaacataaaaattggtcagttgataaatacaaagactgccactgcacgagagtttaataaacaagctt

SEQ ID NO: 24 - DNA, 4321 bp, synthetic construct
  source 1..4321: mol_type = other DNA
cgcaaccaagggctagcaatgtcagtaaagctagtcacctggaccacgagttgccgaagctcgttcagtgtttcagagttaaaaaatgtgttttaaataatttaagaactgcaaatgcaatgctcacttataatttaataattacaattttgcttcctatggcgggcaagggaggtctggttgtcggccatgctggaaatgtgatctcgcgttattgtgccattgtcaatacagtacatctacaccacgatatgaaacgttgatttgaaccttctgactcacttgtgaatcagacgggccccatggtctgatttaaatcgcatgatatctgatgatagttgtcgaatatatcgactgattgcattacctcatccccatactgtatttatttatttatcttgctcctttgcacctcagtatctctacttgcacattcatcttctgcacatctaacattccagtgtttaattgctatattgtaattacttcgccaccatggcctatttattgccttaacgctcttatcttacctcatttgcactcactgcattctttttctactgtattattgactgtatgttttgtttattccatgtgtaactctgtgttgttgtaaatgtcgaactgctatgatttatcttggccaggtcgcagttgcaaatgagaacttgttctcaactaacctacctggttaaataaaggttaaataaaggttaaataaaaaataaataaataaaaagtgtatccggtgcgaacgcaacccgacgtcttcatgggaagtgggagggagcaacagcctgtgtttttattggtattttggaatgtcaagttgaatcctgagctatgattggttgccttgccgtttatatagtaatggtagacttatccttccttctttctctcacaacacacaaggcgaagaaagggaggcttcgccattgttcaactccgatcaacatcagcatcaccttcggtcaaataatttattcggtaagtaagaactagtttaatttaatagtaatgtaataatgaaagcgtttttttttagttcaccgtaatttattttgctgaccacaagccggtacattttatatccggaagacaaggctggctaacgtaaattaactacttggccttgtagttttaactaatatcacctagtcgacaaattaaaccttgtaaaacttacctaactgatctagctttaactcggaattactgcaatatatttacatgttctatcctatttgatatcatttaactgttaacgttgggcaactagttcgcttttagttggcctttgcttgctaactaatcggtcaacctttaatgtcgtggttaatatcacagctaataattatttgattgacattcgatcgacagtttcaaacagtttttgtcactgcgctaggtaacaacggttgtatgcggtataccaggatatggcgcgcgaccaccctcgtggtcggcctagttctagaacgttctagagactctgcaccccgcgtgatgtgacgcacaaaaggacgtccgttgttctttctgaagtgtaataccggtacataccggtatctgttgctgaagttggtgtcgacgtgagcaccgtatcttgaattaaaccgttttattggttagtcgatactttagttttgctgaccttattctcataggctgttcgggggacaaatatttaactttggttgtgttatatcttatgatctctttatagcgatcactattttgagcgaaggacttaaaataagggaagtttattgtttttctagtcaatggtatcaaatcaattgaattaactttttgggcgacctgacggtaattcgcatgcgagttatagagctctcattgaaagtcttaaaagcggtaggtctgatataggtgcgccatttctatgtttccgggtcacaagcttctttctgcttctactttctattttctgaaagtattttcggctttggaaaataatttagtagtttcgatggtgcgaccggtctaccctatagctgttgcataaactgtatttgggaaaatatcagttttggcaaccaggaaatggctgcggtttatgcttagtggctttaaatttaacttgatagtatttcaaaccactaattgactgactttggttcaattatttgaggaatattttcccctgtgagctcagtgcgctcgctgccgtttcttgggtgaaatcagatccagcctgaactgtgccatgtagtgggtagtttgtaacttccaactggccaatttcctacacatttgagaacatgtggtaattaactacaatgactaattggttatctacatttatccctgcccctgaggcaaatggcactatggagtgcctgaggtggcaaaatgtaaatctggaactatccctgacaaccaatgtcaatgtagctacagggttcaacttcgtagaatgatttcatgtctcggaacaatgacaggagtggaggtgttttgctttttcggtgaagatgtcaaatgaccatcaaacaaaatcaggactctaccatactacttgacaatacaatgtcgcatcaatcttactcggttaggttgaagaataccattgtgaatgtgaacacgaatttagcagttttcaaagacctgtcccacattggaaaattcctaggatggtacttgagtctacaatgtgcagttgggcctagaggggtaactaatgtttacaaatgaccaatgtattttgatgaccacattggcttctagctgatatttttactgcgtttgttgtattcttgcatagtgtccatttgttacctaacaccatgctgttcttcattgtccaggtaacatgtctaagggaatgtactgcacccacttaaagatgctgcagctggtcgtcatggcaacgctgtgggtgacaccagtgagggcggggacagactgcaggtatggctgccgactaaacaacatgaccatcaccgtggagagagaggactgtcacggaagcatcaccgtcaccacctgcgccggcctgtgcgaaacaacggacctgaactatcagagcacatggctgccgcgctcccagggggtgtgtaacttcaaggagtggtcctacgagaaggtctacctggaaggctgtccatccggggtcaaccccctcttcatacccgttgccaagagctgcgattgcatcaaatgcaagacggacaacaccgactgtgatcgcataagcatggcaacacccagctgcatagtaaacccactagaaatgtcctcttcctctaaggatccacatcaccatcaccatcacccatcccaacctctcacatccacatccaccccaactcctggggccaacagacgttcctctcatcccctcccaataaagacttcttatccaaacagtgacaagacaaacatgggctgtgaggaatgcacactgaagccgaacacaatcttccccaacatcatgcagtgtacaggctgttgcttctccagagcttatccaaccccactacggtccaagcaaaccatgctggttcccaagaacatcacctctgaagccacatgctgcgttgcaaaagaaggggaaagggtcaccaccaaggatggcttcccggtgacgaaccacacagagtgtcactgcagcacctgctattaccataaatcataaacattccattgtttctgcaactacctccccctaacaagcaaagtttgaaatgtgttctaccctcttgtgtctgagtctcgtgacttgtcaaggagtgaaatttgaataaaggttgggggatcacatatttttcaactttgtttgctacgcaacagggaacagtaattttctgttagcacaactaagctgtcaaatttcacatgtgtattttctcagttgtcatctgcctttgtcacaatgcctttaggacaaaataaaatatacggtgaccttccacctttacttctaaatgtttgggtcctttacactactttggaaaagggaagatgttaggaagggccatattttggtcaatattgtcatgacaaagttcaatattgcttgtagcttcccacaaacttccagctgctagaccagtgtaaagatgtcttgaggtcctgcgtccattcatacctgaccctttttttttgaatgtggtagtgcttcatatctataccattggaaaaacataaattgctttaagtgactaccgagtcattttggtacatttcctcgtgtgcctaaccaaagcaaaaaaggccctggcctatggaaacataaaaattggtcagttgataaatacaaagactgccactgcacgagagtttaataaacaagctt

SEQ ID NO: 25 - DNA, 813 bp, synthetic construct
  source 1..813: mol_type = other DNA
atgtactgcacccacttaaagatgctgcagctggtcgtcatggcaacgctgtgggtgacaccagtgagggcggggacagactgcaggtatggctgccgactaaacaacatgaccatcaccgtggagagagaggactgtcacggaagcatcaccgtcaccacctgcgccggcctgtgcgaaacaacggacctgaactatcagagcacatggctgccgcgctcccagggggtgtgtaacttcaaggagtggtcctacgagaaggtctacctggaaggctgtccatccggggtcaaccccctcttcatacccgttgccaagagctgcgattgcatcaaatgcaagacggacaacaccgactgtgatcgcataagcatggcaacacccagctgcatagtaaacccactagaaatgtcctcttcctctaaggatccacatcaccatcaccatcacccatcccaacctctcacatccacatccaccccaactcctggggccaacagacgttcctctcatcccctcccaataaagacttcttatccaaacagtgacaagacaaacatgggctgtgaggaatgcacactgaagccgaacacaatcttccccaacatcatgcagtgtacaggctgttgcttctccagagcttatccaaccccactacggtccaagcaaaccatgctggttcccaagaacatcacctctgaagccacatgctgcgttgcaaaagaaggggaaagggtcaccaccaaggatggcttcccggtgacgaaccacacagagtgtcactgcagcacctgctattaccataaatcataa

SEQ ID NO: 26 - DNA, 1166 bp, synthetic construct
  source 1..1166: mol_type = other DNA
ttacaaatgaccaatgtattttgatgaccacattggcttctagctgatatttttactgcgtttgttgtattcttgcatagtgtccatttgttacctaacaccatgctgttcttcattgtccaggtaacatgtctaagggaatgtactgcacccacttaaagatgctgcagctggtcgtcatggcaacgctgtgggtgacaccagtgagggcggggacagactgcaggtatggctgccgactaaacaacatgaccatcaccgtggagagagaggactgtcacggaagcatcaccgtcaccacctgcgccggcctgtgcgaaacaacggacctgaactatcagagcacatggctgccgcgctcccagggggtgtgtaacttcaaggagtggtcctacgagaaggtctacctggaaggctgtccatccggggtcaaccccctcttcatacccgttgccaagagctgcgattgcatcaaatgcaagacggacaacaccgactgtgatcgcataagcatggcaacacccagctgcatagtaaacccactagaaatgtcctcttcctctaaggatccacatcaccatcaccatcacccatcccaacctctcacatccacatccaccccaactcctggggccaacagacgttcctctcatcccctcccaataaagacttcttatccaaacagtgacaagacaaacatgggctgtgaggaatgcacactgaagccgaacacaatcttccccaacatcatgcagtgtacaggctgttgcttctccagagcttatccaaccccactacggtccaagcaaaccatgctggttcccaagaacatcacctctgaagccacatgctgcgttgcaaaagaaggggaaagggtcaccaccaaggatggcttcccggtgacgaaccacacagagtgtcactgcagcacctgctattaccataaatcataaacattccattgtttctgcaactacctccccctaacaagcaaagtttgaaatgtgttctaccctcttgtgtctgagtctcgtgacttgtcaaggagtgaaatttgaataaaggttgggggatcacatatttttcaactttgtttgctacgcaacagggaacagtaattttctgttagcacaactaagctgtcaaatttcacatgtgtattttct